European Patent Specification EP 4 150 103 B1, published April 9, 2025. Title: Verfahren zur Herstellung von hydroxyfettsäurebasierten Polyolen. Applicant: U. Windmöller Innovation GmbH & Co. KG Universität Bielefeld. The sequence listing filed with the application follows.

SEQUENCE LISTING (3 sequences)

SEQ ID NO: 1 - DNA, 2022 bp, Artificial Sequence
  Sn-Ohy Rohextrakt
atgggcagcagccatcatcatcatcatcacagcagcggcctggtgccgcgcggcagccatatggaagaagtgagttatcccaaagctggaccgagcattgaagcgaacgtaggggatgggcactggcgaaaggggccctcggatacgctgccgcctccggacactgttggaccctatatgcgcaaccgccccctgcctgtggatcaagtggaaggcaggaaagcatggatcatcggaagtggaatcgcgggtctggcctctgccttttacttgatccgcgacgggcggatgaaggggcaggacataaccatcctcgatgccgtgggcactccaggcggatcactggacggctcagggaacgccgaagatggctacctgatccgaggcgggcgcgagatgaactggaactacgatcacttttgggatctcttccaggacattcccgcgctggagtacccgtccccttactcggtcttggatgagtatcgggcggtgaacgacaatgatcctaattggtccaagtcccgattgatgcacaagcaaggccaaattcgggatttcagcaccttggggctttcttccgcccaccaatgggaattgatcaagcttctcctgaagcgcaaggaggacctcgatgacatcaccatcgaacagtacttcagcgatagctttctggagaccaacttctggtacctctggcgctcgatgtttgcgttccagaactggcaaagtctgctggaagtgaagttgtacatgcatcgctttttggatgcaatcgacggcttgacggatatgtcagcgctcgtgttcccaaaatacaaccagtacgacagcttcgtcgtccccctggtcaactacctcaagggccaaggcgtcaacgtagaattcggcacgcgcgtctacgacctggacatgacggacaacaacggcgagcgtaccgtgacctccattcttgcgaaggtagacgggcgggatcagaagattgacatcggcgcgaaggacgtggtttttgccctgactggatcgatgacggagggtacagcctacggcgatctggatactgctcccgacctcactcgagccaccacgccccctggcgactcaagcgattgggcgttgtggcagaacctggccaagaagtcccacgtctttggtaagcctgaaaagttctgcgggcaacccagtcgctcgatgtgggagtctgccaccctgacgtgcaagccttcgccgttgaccgagcgcctcaaagatctctcaatcaatgacccttattcgggaaaaacggtgaccggtggaatcatcacctttaccgactcgaactgggttctcagcttcacctgcaatcgtcaaccgcatttccccacacaaccagacgacgtactggtgctttgggtctatgccttggtcatggacagcaaaggcaaccatgtactaaaaccaatgcctgagtgtacgggccgcgaaattcttgctgagctttgctaccacctcggcattgtggatcaggtggatgaagtggccagacagaccaaggttcgccttgccctgatgccattcatcacggctcaatttatgccacgagctgctggagatcgaccgcgtgttgttccagccgggtgcaccaatctcgctctgctgggccaattcgtggagacgtctaatgacatcatcttcaccatggagagttccgtcaggactgcgcggattggcgtgtacacgcttctggggctacgaaagcaggtcgccgatatcagccccacgcaatacgacgtccgaaatctgatcaagggtgctcgtgccctgaacaacaacgagccgttcatgggcgagcggctgctccatcgactgctcgacaacacctacttcgcccacatcctcccgccgctgccagcaggagacggtggatccagcgatcaagcggcaagctcgcgtatgaaggccaaccacactgcggcggcggcacttggagcggtgtctgattggatccatcatgttcgggataaactgaagccgggcgcctga

SEQ ID NO: 2 - protein, 673 aa, Artificial Sequence
  Sn-Ohy Rohextrakt
MGSSHHHHHHSSGLVPRGSHMEEVSYPKAGPSIEANVGDGHWRKGPSDTLPPPDTVGPYMRNRPLPVDQVEGRKAWIIGSGIAGLASAFYLIRDGRMKGQDITILDAVGTPGGSLDGSGNAEDGYLIRGGREMNWNYDHFWDLFQDIPALEYPSPYSVLDEYRAVNDNDPNWSKSRLMHKQGQIRDFSTLGLSSAHQWELIKLLLKRKEDLDDITIEQYFSDSFLETNFWYLWRSMFAFQNWQSLLEVKLYMHRFLDAIDGLTDMSALVFPKYNQYDSFVVPLVNYLKGQGVNVEFGTRVYDLDMTDNNGERTVTSILAKVDGRDQKIDIGAKDVVFALTGSMTEGTAYGDLDTAPDLTRATTPPGDSSDWALWQNLAKKSHVFGKPEKFCGQPSRSMWESATLTCKPSPLTERLKDLSINDPYSGKTVTGGIITFTDSNWVLSFTCNRQPHFPTQPDDVLVLWVYALVMDSKGNHVLKPMPECTGREILAELCYHLGIVDQVDEVARQTKVRLALMPFITAQFMPRAAGDRPRVVPAGCTNLALLGQFVETSNDIIFTMESSVRTARIGVYTLLGLRKQVADISPTQYDVRNLIKGARALNNNEPFMGERLLHRLLDNTYFAHILPPLPAGDGGSSDQAASSRMKANHTAAAALGAVSDWIHHVRDKLKPGA

SEQ ID NO: 3 - DNA, 60 bp, Artificial Sequence
  N-terminaler His6-Tag (pET28-Sn-Ohy(N)His6)
atgggcagcagccatcatcatcatcatcacagcagcggcctggtgccgcgcggcagccat